European Patent Specification EP 3 914 620 B1, published November 26, 2025. Title: TREATMENT OF T CELL LYMPHOMA. Applicant: Innate Pharma. The sequence listing filed with the application follows.

SEQUENCE LISTING (70 sequences)

SEQ ID NO: 1 - protein, 434 aa, homo sapiens
LMGGQDKPFLSARPSTVVPRGGHVALQCHYRRGFNNFMLYKEDRSHVPIFHGRIFQESFIMGPVTPAHAGTYRCRGSRPHSLTGWSAPSNPLVIMVTGNHRKPSLLAHPGPLLKSGETVILQCWSDVMFEHFFLHRDGISEDPSRLVGQIHDGVSKANFSIGPLMPVLAGTYRCYGSVPHSPYQLSAPSDPLDIVITGLYEKPSLSAQPGPTVQAGENVTLSCSSWSSYDIYHLSREGEAHERRLRAVPKVNRTFQADFPLGPATHGGTYRCFGSFRALPCVWSNSSDPLLVSVTGNPSSSWPSPTEPSSKSGICRHLHVLIGTSVVIFLFILLLFFLLYRWCSNKKNAAVMDQEPAGDRTVNRQDSDEQDPQEVTYAQLDHCVFIQRKISRPSQRPKTPLTDTSVYTELPNAEPRSKVVSCPRAPQSGLEGVF

SEQ ID NO: 2 - protein, 455 aa, homo sapiens [sequence omitted]

SEQ ID NO: 3 - protein, 123 aa, mus musculus
QVQLKESGPGLVAPSQSLSITCTVSGFSLTSFGVHWVRQPPGKGLEWLGVIWAGGSTNYNSALMSRLSISKDNSKSQVFLKMNSLQNDDTAMYYCARGNSNHYVSSFYYFDYWGQGTTLTVSS

SEQ ID NO: 4 - protein, 106 aa, mus musculus
DIQMTQSPSSLSASLGGKVTITCKASQDINKYIAWYQHKPGKGPRLLIHYTSTLQPGIPSRFSGSGSGRDYSFSISNLEPEDITTYYCLQYDNLWTFGGGTKLEIK

SEQ ID NO: 5 - protein, 119 aa, mus musculus
QIQLVQSGPELKKPGETVKISCKASGYTFTNFGMNWVKQAPGKGLKWMGWINTYTGEPTYADDFKGRFAFSLETSASTAYLQINNLKNEDMATYFCARNGNFGYYFDYWGQGTTLTVSS

SEQ ID NO: 6 - protein, 112 aa, mus musculus
DVLMTQTPLSLPVSLGDQASFSCRSSQNIVHSNGNTYLEWYLQKPGQSPSLLIYKVSNRFSGVPDRFSGSGSGTDFTLKITRVEAEDLGVYYCFQGSHVPFTFGSGTKLEIK

SEQ ID NO: 7 - protein, 5 aa, mus musculus
NFGMN

SEQ ID NO: 8 - protein, 6 aa, mus musculus
GYTFTN

SEQ ID NO: 9 - protein, 10 aa, mus musculus
GYTFTNFGMN

SEQ ID NO: 10 - protein, 15 aa, Mus musculus
WINTYTGEPTYADDF

SEQ ID NO: 11 - protein, 8 aa, Mus musculus
WINTYTGE

SEQ ID NO: 12 - protein, 10 aa, Mus musculus
NGNFGYYFDY

SEQ ID NO: 13 - protein, 16 aa, Mus musculus
RSSQNIVHSNGNTYLE

SEQ ID NO: 14 - protein, 7 aa, Mus musculus
KVSNRFS

SEQ ID NO: 15 - protein, 7 aa, Mus musculus
KVSNRFS

SEQ ID NO: 16 - protein, 112 aa, Mus musculus
QLVQSGPELKNPGETVKISCKASGYTFTNYGMNWVKQAPGKGLKWMGWINTYTGEPTYADDFKGRFAFSLETSASTAYLQINNLKNEDTATYFCAHGPWLAYWGQGTLVTVS

SEQ ID NO: 17 - protein, 107 aa, Mus musculus
DIKMTQSPSSMYASLGERVTITCKASQDINVYLSWFQQKPGKSPKTLIYRAIRLVDGVPSRFSGSGSGQDYSLTISSLDYEDMGIYYCLQYDELPYTFGGGTKLEIE

SEQ ID NO: 18 - protein, 5 aa, Mus musculus
NYGMN

SEQ ID NO: 19 - protein, 6 aa, Mus musculus
GYTFTN

SEQ ID NO: 20 - protein, 10 aa, Mus musculus
GYTFTNYGMN

SEQ ID NO: 21 - protein, 17 aa, Mus musculus
WINTYTGEPTYADDFKG

SEQ ID NO: 22 - protein, 10 aa, Mus musculus
WINTYTGEPT

SEQ ID NO: 23 - protein, 6 aa, Mus musculus
GPWLAY

SEQ ID NO: 24 - protein, 11 aa, Mus musculus
KASQDINVYLS

SEQ ID NO: 25 - protein, 7 aa, Mus musculus
RAIRLVD

SEQ ID NO: 26 - protein, 9 aa, Mus musculus
LQYDELPYT

SEQ ID NO: 27 - protein, 117 aa, Mus musculus
QIQLVQSGPELKKPGETVRISCKASGYTFTIAGMQWVQKMPGKGLKWIGWINTHSGVPKYAEDFKGRFAFSLETSANIAYLQISNLKNEDTATYFCARGGDEGVMDYWGQGTSVTVS

SEQ ID NO: 28 - protein, 107 aa, Mus musculus
DIVMTQSHKFMSTSVGDRVSITCKASQDVSTAVAWYHQKPGQSPKLLIYWASTRHTGVPDRFSGSGSGTDYTLTISALQAEDLALYYCQQHYNTPWTFGGGTKLEIK

SEQ ID NO: 29 - protein, 120 aa, Mus musculus
QVQLQQSAAELARPGASVKMSCKASGYTFTSYTMHWVKQRPGQGLEWIGYINPSSGYTDYNQKFKDKTTLTADRSSSTAYMQLSSLTSEDSAVYYCARLGKGLLPPFDYWGQGSTLTVSS

SEQ ID NO: 30 - protein, 113 aa, Mus musculus
EIVLTQSIPSLTVSAGERVTISCKSNQNLLWSGNQRYCLVWHQWKPGQTPTPLITWTSDRYSGVPDRFIGSGSVTDFTLTISSVQAEDVAVYFCQQHLHIPYTFGGGTKLEIK

SEQ ID NO: 31 - protein, 119 aa, Mus musculus
EVQLQQSGPELVKPGASMKISCKASHYSFIGYTMNWVKQRHGKNLEWIGLINPYNGDTTYNQKFKGKASLTVDKSSSTAYMEILSLTSEDSAVYYCARENWGYPYAMDYWGQGTSVTVS

SEQ ID NO: 32 - protein, 117 aa, Mus musculus
QIQLVQSGPELKKPGETVRISCKASGYTFTTAGMQWVQKTPGKGLKWIGWINSHSGVPKYAEDFKGRFAFSLETSASTAYLQISTLKNEDTATYFCARGGDEGVMDYWGQGTSVTVS

SEQ ID NO: 33 - protein, 107 aa, Mus musculus
DIVMTQSHKFMSTSLGDRVSFTCKASQDVSTAVAWYQQKPGQSPKLLIYWTSTRHTGVPDRFTGSGSGTDYTLTISSVQAEDLALYYCQQHYSTPWTFGGGTKLEIK

SEQ ID NO: 34 - protein, 6 aa, Mus musculus
GYTFTT

SEQ ID NO: 35 - protein, 5 aa, Mus musculus
TAGMQ

SEQ ID NO: 36 - protein, 10 aa, Mus musculus
GYTFTTAGMQ

SEQ ID NO: 37 - protein, 17 aa, Mus musculus
WINSHSGVPKYAEDFKG

SEQ ID NO: 38 - protein, 9 aa, Mus musculus
WINSHSGVP

SEQ ID NO: 39 - protein, 9 aa, Mus musculus
GGDEGVMDY

SEQ ID NO: 40 - protein, 11 aa, Mus musculus
KASQDVSTAVA

SEQ ID NO: 41 - protein, 7 aa, Mus musculus
WTSTRHT

SEQ ID NO: 42 - protein, 9 aa, Mus musculus
QQHYSTPWT

SEQ ID NO: 43 - protein, 107 aa, Artificial
  Synthetic
DIQMTQSPSFLSASVGDRVTITCKASQDVSTAVAWYQQKPGQPPKLLIYWTSTRHTGVPDRFSGSGSGTDFTLTISSLQAEDVAVYYCQQHYSTPWTFGGGTKVEIK

SEQ ID NO: 44 - protein, 107 aa, Artificial
  Synthetic
DIQMTQSPSFLSASVGDRVTITCKASQDVSTAVAWYQQKPGQPPKLLIYWTSTRHTGVPDRFSGSGSGTDYTLTISSLQAEDVAVYYCQQHYSTPWTFGGGTKVEIK

SEQ ID NO: 45 - protein, 107 aa, Artificial
  Synthetic
DIVMTQSPSFLSASVGDRVTITCKASQDVSTAVAWYQQKPGQPPKLLIYWTSTRHTGVPDRFSGSGSGTDYTLTISSVQAEDVAVYYCQQHYSTPWTFGGGTKVEIK

SEQ ID NO: 46 - protein, 107 aa, Artificial
  Synthetic
DIVMTQSPSFLSASVGDRVTFTCKASQDVSTAVAWYQQKPGQSPKLLIYWTSTRHTGVPDRFSGSGSGTDYTLTISSVQAEDVAVYYCQQHYSTPWTFGGGTKVEIK

SEQ ID NO: 47 - protein, 107 aa, Artificial
  Synthetic
DIVMTQSHKFLSASVGDRVTFTCKASQDVSTAVAWYQQKPGQSPKLLIYWTSTRHTGVPDRFSGSGSGTDYTLTISSVQAEDVAVYYCQQHYSTPWTFGGGTKLEIK

SEQ ID NO: 48 - protein, 118 aa, Artificial
  Synthetic
QVQLVQSGSELKKPGASVKVSCKASGYTFTTAGMQWVQKSPGQGLEWMGWINSHSGVPKYAEDFKGRFVFSLDTSVSTAYLQISSLKAEDTAVYFCARGGDEGVMDYWGQGTTVTVSS

SEQ ID NO: 49 - protein, 118 aa, Artificial
  Synthetic
QIQLVQSGSELKKPGASVKVSCKASGYTFTTAGMQWVRQAPGQGLEWIGWINSHSGVPKYAEDFKGRFVFSLDTSVSTAYLQISSLKAEDTAVYFCARGGDEGVMDYWGQGTTVTVSS

SEQ ID NO: 50 - protein, 118 aa, Artificial
  Synthetic
QIQLVQSGSELKKPGASVKVSCKASGYTFTTAGMQWVQKSPGQGLEWIGWINSHSGVPKYAEDFKGRFAFSLDTSVSTAYLQISSLKAEDTAVYFCARGGDEGVMDYWGQGTTVTVSS

SEQ ID NO: 51 - protein, 118 aa, Artificial
  Synthetic
QIQLVQSGSELKKPGASVKVSCKASGYTFTTAGMQWVQKTPGKGLEWIGWINSHSGVPKYAEDFKGRFAFSLDTSASTAYLQISSLKAEDTAVYFCARGGDEGVMDYWGQGTSVTVSS

SEQ ID NO: 52 - protein, 107 aa, Artificial
  Synthetic
DIQMTQSPSSLSASVGDRVTITCRASENIYSNLAWYQQKPGKAPKLLLYAATNLADGVPSRFSGSGSGTDYTLTISSLQPEDFATYYCQHFWGTPYTFGQGTKLEIK

SEQ ID NO: 53 - protein, 107 aa, Artificial
  Synthetic
DIQMTQSPSSLSASVGDRVTITCRASENIYSNLAWYQQKPGKAPQLLVYAATNLADGVPSRFSGSGSGTDYTLTISSLQPEDFATYYCQHFWGTPYTFGGGTKLEIK

SEQ ID NO: 54 - protein, 107 aa, Artificial
  Synthetic
DIQMTQSPSSLSASVGDRVTITCRASENIYSNLAWYQQKPGKAPQLLVYAATNLADGVPSRFSGSGSGTQYTLTISSLQPEDFATYYCQHFWGTPYTFGGGTKLEIK

SEQ ID NO: 55 - protein, 107 aa, Artificial
  Synthetic
DIQMTQSPSSLSASVGDRVTITCRASENIYSNLAWYQQKQGKAPQLLVYAATNLADGVPSRFSGSGSGTQYTLTINSLQPEDFATYYCQHFWGTPYTFGGGTKLEIK

SEQ ID NO: 56 - protein, 107 aa, Artificial
  Synthetic
DIQMTQSPSSLSASVGETVTITCRASENIYSNLAWYQQKQGKAPQLLVYAATNLADGVPSRFSGSGSGTQYTLTINSLQPEDFATYYCQHFWGTPYTFGGGTKLEIK

SEQ ID NO: 57 - protein, 120 aa, Artificial
  Synthetic
QVQLVQSGAEVKKPGASVKVSCKASGYTFTSYTMHWVRQAPGQGLEWMGYINPSSGYTENNRKFKDRVTMTRDTSTSTVYMELSSLRSEDTAVYYCARLGKGLLPPFDYWGQGTTVTVSS

SEQ ID NO: 58 - protein, 120 aa, Artificial
  Synthetic
QVQLVQSGAEVKKPGASVKVSCKASGYTFTSYTMHWVRQAPGQGLEWIGYINPSSGYTENNRKFKDKTTMTADTSTSTAYMELSSLRSEDTAVYYCARLGKGLLPPFDYWGQGTTVTVSS

SEQ ID NO: 59 - protein, 120 aa, Artificial
  Synthetic
QVQLQQSGAEVKKPGASVKMSCKASGYTFTSYTMHWVRQAPGQGLEWIGYINPSSGYTENNRKFKDKTTLTADTSTSTAYMELSSLRSEDTAVYYCARLGKGLLPPFDYWGQGTTLTVSS

SEQ ID NO: 60 - protein, 120 aa, Artificial
  Synthetic
QVQLVQSGAELARPGASVKVSCKASGYTFTSYTMHWVRQAPGQGLEWIGYINPSSGYTENNRKFKDKTTLTADKSTSTAYMELSSLRSEDTAVYYCARLGKGLLPPFDYWGQGTTVTVSS

SEQ ID NO: 61 - protein, 120 aa, Artificial
  Synthetic
QVQLQQSGAEVKKPGASVKMSCKASGYTFTSYTMHWVKQRPGQGLEWIGYINPSSGYTENNRKFKDKTTLTADKSTSTAYMELSSLRSEDTAVYYCARLGKGLLPPFDYWGQGTTLTVSS

SEQ ID NO: 62 - protein, 111 aa, Mus musculus
DIVLTQSPASLAVSLGQRATISCRASESVDNFGISFMNWFQQKPGQPPKLLIYAASNQGSGVPARFSGSRSGTDFSLNIHPMEEDDTAMYFCQQSKEVPYTFGGGTKLEIK

SEQ ID NO: 63 - protein, 117 aa, Mus musculus
QVQLQQSGAELVRPGVSVKISCKGSGYTFTDYAMNWVKQSHAKSLEWIGVISTYYGDANYNQKFKGKATMTVDKSSSTAYMELARLTSEDSAIYYCALIYYDYDGSYWGQGTTLTVS

SEQ ID NO: 64 - protein, 113 aa, Mus musculus
DVVMTQTPLSLPVSLGDQASISCRSSQSLVHSNGNTYLHWYLQKPGQSPKLLIYKVSNRFSGVPDRFSGSGSGTDFTLKISRVEAEDLGVYFCSQSTHVPPYTFGGGTKLEIK

SEQ ID NO: 65 - protein, 118 aa, Mus musculus
QVQLQQSGAELARPGASVKLSCKASGYTFTSYWMQWVKQRPGQGLEWIGAIYPGDGDTRYTQKFKGKATLTADKSSSTAYMQLSSLASEDSAVYYCARRYDGYYHFDYWGQGTTLTVS

SEQ ID NO: 66 - protein, 115 aa, Mus musculus
DIVMTQSPSSLAVTAGEKVTMSCKSSQSLLWSVNQKNYLSWYQQKQRQPPKLLIYGASIRESWVPDRFTGSGSGTDFTLTISNVHAEDLAVYYCQHNHGSFLPLTFGSGTKLEIK

SEQ ID NO: 67 - protein, 120 aa, Mus musculus
QVQLQQSGAEVARPGASVKLSCKSSGFTFTTYWMQWVKQRPGQGLEWIGAIYPGDGDTRYTQKFKGKATLTADKSSITAYMQLSSLASEDSAVYYCARRGDYGNYGMDYWGQGTSVTVSS

SEQ ID NO: 68 - protein, 112 aa, Mus musculus
DVLMTQTPLSLPVSLGDQASISCRSSQSIVHSNGNTYLEWYLQKPGQSPKLLIYKVSNHFSGVPDRFSGSGSGTDFTLKISRVEAEDLGVYYCFQGSHVPPTFGGGTKLEIK

SEQ ID NO: 69 - protein, 139 aa, Mus musculus
QVQLQQSAAELARPGASVKMSCKASGYTFTSYTMHWVKQRPGQGLEWIGYINPSSGYTENNRKFKDKTTLTADKSSSTAYMQLSSLTSEDSAVYYCARLGKGLLPPFDYWGQGTTLTVSSAKTTPPSVYPLAPGSAAQT

SEQ ID NO: 70 - protein, 107 aa, mus musculus
DIQMTQSPASLSVSVGETVTITCRASENIYSNLAWYQQKQGKSPQLLVYAATNLADGVPSRFSGSGSGTQYSLKINSLQSEDFGSYYCQHFWGTPYTFGGGTKLEIK